European Patent Application EP 4 183 419 A1, published May 24, 2023. Title: Therapeutic use of a combination comprising triple agonistic long-acting conjugate or triple agonist. Applicant: HANMI PHARM. CO., LTD. The sequence listing filed with the application follows.

SEQUENCE LISTING (139 sequences)

SEQ ID NO: 1 - protein, 30 aa, Artificial Sequence
  Trigonal agonist
  MISC_FEATURE (2): Xaa is 2-aminoisobutyric acid (Aib)
HXQGTFTSDVSSYLDGQAAKEFIAWLVKGC

SEQ ID NO: 2 - protein, 30 aa, Artificial Sequence
  Trigonal agonist
  MISC_FEATURE (2): Xaa is 2-aminoisobutyric acid (Aib)
HXQGTFTSDVSSYLDGQAQKEFIAWLVKGC

SEQ ID NO: 3 - protein, 41 aa, Artificial Sequence
  Trigonal agonist
  MISC_FEATURE (2): Xaa is 2-aminoisobutyric acid (Aib)
HXQGTFTSDVSSYLLGQAAKQFIAWLVKGGGPSSGAPPPSC

SEQ ID NO: 4 - protein, 30 aa, Artificial Sequence
  Trigonal agonist
  MISC_FEATURE (2): Xaa is 2-aminoisobutyric acid (Aib)
HXQGTFTSDVSSYLLGQQQKEFIAWLVKGC

SEQ ID NO: 5 - protein, 41 aa, Artificial Sequence
  Trigonal agonist
  MISC_FEATURE (2): Xaa is 2-aminoisobutyric acid (Aib)
HXQGTFTSDVSSYLLGQQQKEFIAWLVKGGGPSSGAPPPSC

SEQ ID NO: 6 - protein, 30 aa, Artificial Sequence
  Trigonal agonist
  MISC_FEATURE (2): Xaa is 2-aminoisobutyric acid (Aib)
HXQGTFTSDVSSYLDGQAAKEFVAWLLKGC

SEQ ID NO: 7 - protein, 30 aa, Artificial Sequence
  Trigonal agonist
  MISC_FEATURE (2): Xaa is 2-aminoisobutyric acid (Aib)
HXQGTFTSDVSKYLDGQAAKEFVAWLLKGC

SEQ ID NO: 8 - protein, 30 aa, Artificial Sequence
  Trigonal agonist
  MISC_FEATURE (2): Xaa is 2-aminoisobutyric acid (Aib)
HXQGTFTSDVSKYLDGQAAQEFVAWLLKGC

SEQ ID NO: 9 - protein, 30 aa, Artificial Sequence
  Trigonal agonist
  MISC_FEATURE (2): Xaa is 2-aminoisobutyric acid (Aib)
HXQGTFTSDVSKYLDGQAAQEFVAWLLAGC

SEQ ID NO: 10 - protein, 41 aa, Artificial Sequence
  Trigonal agonist
  MISC_FEATURE (2): Xaa is 2-aminoisobutyric acid (Aib)
HXQGTFTSDVSKYLDGQAAQEFVAWLLAGGGPSSGAPPPSC

SEQ ID NO: 11 - protein, 41 aa, Artificial Sequence
  Trigonal agonist
  MISC_FEATURE (1): Xaa is 4-imidazoacetyl (CA)
XGEGTFTSDLSKYLDSRRQQLFVQWLKAGGPSSGAPPPSHG

SEQ ID NO: 12 - protein, 41 aa, Artificial Sequence
  Trigonal agonist
  MISC_FEATURE (1): Xaa is 4-imidazoacetyl (CA)
XGEGTFISDLSKYMDEQAVQLFVEWLMAGGPSSGAPPPSHG

SEQ ID NO: 13 - protein, 41 aa, Artificial Sequence
  Trigonal agonist
  MISC_FEATURE (1): Xaa is 4-imidazoacetyl (CA)
XGEGTFISDYSIQLDEIAVQDFVEWLLAQKPSSGAPPPSHG

SEQ ID NO: 14 - protein, 41 aa, Artificial Sequence
  Trigonal agonist
  MISC_FEATURE (1): Xaa is 4-imidazoacetyl (CA)
XGQGTFTSDYSIQLDEIAVRDFVEWLKNGGPSSGAPPPSHG

SEQ ID NO: 15 - protein, 41 aa, Artificial Sequence
  Trigonal agonist
  MISC_FEATURE (1): Xaa is 4-imidazoacetyl (CA)
XGQGTFTSDLSKQMDEEAVRLFIEWLKNGGPSSGAPPPSHG

SEQ ID NO: 16 - protein, 41 aa, Artificial Sequence
  Trigonal agonist
  MISC_FEATURE (1): Xaa is 4-imidazoacetyl (CA)
XGQGTFTSDLSKQMDSEAQQLFIEWLKNGGPSSGAPPPSHG

SEQ ID NO: 17 - protein, 41 aa, Artificial Sequence
  Trigonal agonist
  MISC_FEATURE (1): Xaa is 4-imidazoacetyl (CA)
XGQGTFTSDLSKQMDEERAREFIEWLLAQKPSSGAPPPSHG

SEQ ID NO: 18 - protein, 41 aa, Artificial Sequence
  Trigonal agonist
  MISC_FEATURE (1): Xaa is 4-imidazoacetyl (CA)
XGQGTFTSDLSKQMDSERAREFIEWLKNTGPSSGAPPPSHG

SEQ ID NO: 19 - protein, 41 aa, Artificial Sequence
  Trigonal agonist
  MISC_FEATURE (1): Xaa is 4-imidazoacetyl (CA)
XGQGTFTSDLSIQYDSEHQRDFIEWLKDTGPSSGAPPPSHG

SEQ ID NO: 20 - protein, 41 aa, Artificial Sequence
  Trigonal agonist
  MISC_FEATURE (1): Xaa is 4-imidazoacetyl (CA)
XGQGTFTSDLSIQYEEEAQQDFVEWLKDTGPSSGAPPPSHG

SEQ ID NO: 21 - protein, 39 aa, Artificial Sequence
  Trigonal agonist
  MISC_FEATURE (2): Xaa is 2-aminoisobutyric acid (Aib)
  MISC_FEATURE (16)..(20): amino acids at positions 16 and 20 form a ring
YXQGTFTSDYSKYLDECRAKEFVQWLLDHHPSSGQPPPS

SEQ ID NO: 22 - protein, 39 aa, Artificial Sequence
  Trigonal agonist
  MISC_FEATURE (2): Xaa is 2-aminoisobutyric acid (Aib)
  MISC_FEATURE (16)..(20): amino acids at positions 16 and 20 form a ring
YXQGTFTSDYSKCLDEKRAKEFVQWLLDHHPSSGQPPPS

SEQ ID NO: 23 - protein, 41 aa, Artificial Sequence
  Trigonal agonist
  MISC_FEATURE (2): Xaa is 2-aminoisobutyric acid (Aib)
  MISC_FEATURE (16)..(20): amino acids at positions 16 and 20 form a ring
YXQGTFTSDYSKYLDECRAKEFVQWLLAQKGKKNDWKHNIT

SEQ ID NO: 24 - protein, 39 aa, Artificial Sequence
  Trigonal agonist
  MISC_FEATURE (2): Xaa is 2-aminoisobutyric acid (Aib)
  MISC_FEATURE (16)..(20): amino acids at positions 16 and 20 form a ring
YXQGTFTSDYSKYLDECRAKEFVQWLKNGGPSSGAPPPS

SEQ ID NO: 25 - protein, 39 aa, Artificial Sequence
  Trigonal agonist
  MISC_FEATURE (2): Xaa is 2-aminoisobutyric acid (Aib)
HXQGTFTSDCSKYLDERAAQDFVQWLLDGGPSSGAPPPS

SEQ ID NO: 26 - protein, 39 aa, Artificial Sequence
  Trigonal agonist
  MISC_FEATURE (2): Xaa is 2-aminoisobutyric acid (Aib)
HXQGTFTSDCSKYLDSRAAQDFVQWLLDGGPSSGAPPPS

SEQ ID NO: 27 - protein, 40 aa, Artificial Sequence
  Trigonal agonist
  MISC_FEATURE (2): Xaa is 2-aminoisobutyric acid (Aib)
HXQGTFTSDYSKYLDERACQDFVQWLLDQGGPSSGAPPPS

SEQ ID NO: 28 - protein, 41 aa, Artificial Sequence
  Trigonal agonist
  MISC_FEATURE (2): Xaa is 2-aminoisobutyric acid (Aib)
HXQGTFTSDYSKYLDEKRAQEFVCWLLAQKGKKNDWKHNIT

SEQ ID NO: 29 - protein, 30 aa, Artificial Sequence
  Trigonal agonist
  MISC_FEATURE (2): Xaa is 2-aminoisobutyric acid (Aib)
  MISC_FEATURE (16)..(20): amino acids at positions 16 and 20 form a ring
HXQGTFTSDYSKYLDEKAAKEFVQWLLNTC

SEQ ID NO: 30 - protein, 30 aa, Artificial Sequence
  Trigonal agonist
  MISC_FEATURE (2): Xaa is 2-aminoisobutyric acid (Aib)
  MISC_FEATURE (16)..(20): amino acids at positions 16 and 20 form a ring
HXQGTFTSDYSKYLDEKAQKEFVQWLLDTC

SEQ ID NO: 31 - protein, 29 aa, Artificial Sequence
  Trigonal agonist
  MISC_FEATURE (2): Xaa is 2-aminoisobutyric acid (Aib)
  MISC_FEATURE (16)..(20): amino acids at positions 16 and 20 form a ring
HXQGTFTSDYSKYLDEKACKEFVQWLLAQ

SEQ ID NO: 32 - protein, 39 aa, Artificial Sequence
  Trigonal agonist
  MISC_FEATURE (2): Xaa is 2-aminoisobutyric acid (Aib)
  MISC_FEATURE (16)..(20): amino acids at positions 16 and 20 form a ring
HXQGTFTSDYSKYLDEKACKDFVQWLLDGGPSSGAPPPS

SEQ ID NO: 33 - protein, 31 aa, Artificial Sequence
  Trigonal agonist
  MISC_FEATURE (2): Xaa is 2-aminoisobutyric acid (Aib)
  MISC_FEATURE (16)..(20): amino acids at positions 16 and 20 form a ring
HXQGTFTSDYSIAMDEIHQKDFVNWLLAQKC

SEQ ID NO: 34 - protein, 31 aa, Artificial Sequence
  Trigonal agonist
  MISC_FEATURE (2): Xaa is 2-aminoisobutyric acid (Aib)
  MISC_FEATURE (16)..(20): amino acids at positions 16 and 20 form a ring
HXQGTFTSDYSKYLDEKRQKEFVNWLLAQKC

SEQ ID NO: 35 - protein, 31 aa, Artificial Sequence
  Trigonal agonist
  MISC_FEATURE (2): Xaa is 2-aminoisobutyric acid (Aib)
  MISC_FEATURE (16)..(20): amino acids at positions 16 and 20 form a ring
HXQGTFTSDYSIAMDEIHQKDFVNWLLNTKC

SEQ ID NO: 36 - protein, 40 aa, Artificial Sequence
  Trigonal agonist
  MISC_FEATURE (2): Xaa is 2-aminoisobutyric acid (Aib)
  MISC_FEATURE (16)..(20): amino acids at positions 16 and 20 form a ring
HXQGTFTSDYSKYLCEKRQKEFVQWLLNGGPSSGAPPPSG

SEQ ID NO: 37 - protein, 40 aa, Artificial Sequence
  Trigonal agonist
  MISC_FEATURE (2): Xaa is 2-aminoisobutyric acid (Aib)
  MISC_FEATURE (16)..(20): amino acids at positions 16 and 20 form a ring
HXQGTFTSDYSKYLDECRQKEFVQWLLNGGPSSGAPPPSG

SEQ ID NO: 38 - protein, 40 aa, Artificial Sequence
  Trigonal agonist
  MISC_FEATURE (1): Xaa is 4-imidazoacetyl (CA)
  MISC_FEATURE (2): Xaa is 2-aminoisobutyric acid (Aib)
XXQGTFTSDKSSYLDERAAQDFVQWLLDGGPSSGAPPPSS

SEQ ID NO: 39 - protein, 40 aa, Artificial Sequence
  Trigonal agonist
  MISC_FEATURE (2): Xaa is 2-aminoisobutyric acid (Aib)
HXQGTFTSDYSKYLDGQHAQCFVAWLLAGGGPSSGAPPPS

SEQ ID NO: 40 - protein, 39 aa, Artificial Sequence
  Trigonal agonist
  MISC_FEATURE (2): Xaa is 2-aminoisobutyric acid (Aib)
HXQGTFTSDKSKYLDERACQDFVQWLLDGGPSSGAPPPS

SEQ ID NO: 41 - protein, 39 aa, Artificial Sequence
  Trigonal agonist
  MISC_FEATURE (2): Xaa is 2-aminoisobutyric acid (Aib)
HXQGTFTSDKSKYLDECAAQDFVQWLLDGGPSSGAPPPS

SEQ ID NO: 42 - protein, 40 aa, Artificial Sequence
  Trigonal agonist
  MISC_FEATURE (2): Xaa is 2-aminoisobutyric acid (Aib)
  MISC_FEATURE (16)..(20): amino acids at positions 16 and 20 form a ring
YXQGTFTSDYSKYLDEKRAKEFVQWLLDHHPSSGQPPPSC

SEQ ID NO: 43 - protein, 39 aa, Artificial Sequence
  Trigonal agonist
  MISC_FEATURE (2): Xaa is 2-aminoisobutyric acid (Aib)
  MISC_FEATURE (16)..(20): amino acids at positions 16 and 20 form a ring
YXQGTFTSDYSKYLDEKRAKEFVQWLLDHHCSSGQPPPS

SEQ ID NO: 44 - protein, 39 aa, Artificial Sequence
  Trigonal agonist
HGQGTFTSDCSKQLDGQAAQEFVAWLLAGGPSSGAPPPS

SEQ ID NO: 45 - protein, 39 aa, Artificial Sequence
  Trigonal agonist
HGQGTFTSDCSKYMDGQAAQDFVAWLLAGGPSSGAPPPS

SEQ ID NO: 46 - protein, 39 aa, Artificial Sequence
  Trigonal agonist
HGQGTFTSDCSKYLDEQHAQEFVAWLLAGGPSSGAPPPS

SEQ ID NO: 47 - protein, 39 aa, Artificial Sequence
  Trigonal agonist
HGQGTFTSDCSKYLDGQRAQEFVAWLLAGGPSSGAPPPS

SEQ ID NO: 48 - protein, 39 aa, Artificial Sequence
  Trigonal agonist
HGQGTFTSDCSKYLDGQRAQDFVNWLLAGGPSSGAPPPS

SEQ ID NO: 49 - protein, 30 aa, Artificial Sequence
  Trigonal agonist
  MISC_FEATURE (1): Xaa is 4-imidazoacetyl (CA)
  MISC_FEATURE (2): Xaa is 2-aminoisobutyric acid (Aib)
  MISC_FEATURE (16)..(20): amino acids at positions 16 and 20 form a ring
XXQGTFTSDYSICMDEIHQKDFVNWLLNTK

SEQ ID NO: 50 - protein, 40 aa, Artificial Sequence
  Trigonal agonist
  MISC_FEATURE (2): Xaa is 2-aminoisobutyric acid (Aib)
  MISC_FEATURE (16)..(20): amino acids at positions 16 and 20 form a ring
HXQGTFTSDYSKYLDEKRAKEFVQWLLDHHPSSGQPPPSC

SEQ ID NO: 51 - protein, 30 aa, Artificial Sequence
  Trigonal agonist
  MISC_FEATURE (2): Xaa is 2-aminoisobutyric acid (Aib)
  MISC_FEATURE (16)..(20): amino acids at positions 16 and 20 form a ring
HXQGTFTSDYSKYLDEKRQKEFVQWLLNTC

SEQ ID NO: 52 - protein, 30 aa, Artificial Sequence
  Trigonal agonist
  MISC_FEATURE (2): Xaa is 2-aminoisobutyric acid (Aib)
  MISC_FEATURE (16)..(20): amino acids at positions 16 and 20 form a ring
HXQGTFTSDYSKYLDEKRQKEFVQWLLDTC

SEQ ID NO: 53 - protein, 30 aa, Artificial Sequence
  Trigonal agonist
  MISC_FEATURE (2): Xaa is 2-aminoisobutyric acid (Aib)
  MISC_FEATURE (16)..(20): amino acids at positions 16 and 20 form a ring
HXEGTFTSDYSIAMDEIHQKDFVNWLLAQC

SEQ ID NO: 54 - protein, 30 aa, Artificial Sequence
  Trigonal agonist
  MISC_FEATURE (2): Xaa is 2-aminoisobutyric acid (Aib)
  MISC_FEATURE (16)..(20): amino acids at positions 16 and 20 form a ring
HXEGTFTSDYSIAMDEIHQKDFVDWLLAEC

SEQ ID NO: 55 - protein, 30 aa, Artificial Sequence
  Trigonal agonist
  MISC_FEATURE (2): Xaa is 2-aminoisobutyric acid (Aib)
  MISC_FEATURE (16)..(20): amino acids at positions 16 and 20 form a ring
HXQGTFTSDYSIAMDEIHQKDFVNWLLAQC

SEQ ID NO: 56 - protein, 30 aa, Artificial Sequence
  Trigonal agonist
  MISC_FEATURE (2): Xaa is 2-aminoisobutyric acid (Aib)
  MISC_FEATURE (16)..(20): amino acids at positions 16 and 20 form a ring
HXQGTFTSDYSKYLDEKRQKEFVNWLLAQC

SEQ ID NO: 57 - protein, 30 aa, Artificial Sequence
  Trigonal agonist
  MISC_FEATURE (2): Xaa is 2-aminoisobutyric acid (Aib)
  MISC_FEATURE (16)..(20): amino acids at positions 16 and 20 form a ring
HXQGTFTSDYSIAMDEIHQKDFVNWLLNTC

SEQ ID NO: 58 - protein, 31 aa, Artificial Sequence
  Trigonal agonist
  MISC_FEATURE (2): Xaa is 2-aminoisobutyric acid (Aib)
  MISC_FEATURE (16)..(20): amino acids at positions 16 and 20 form a ring
HXQGTFTSDYSKYLDEKRQKEFVQWLLNTKC

SEQ ID NO: 59 - protein, 30 aa, Artificial Sequence
  Trigonal agonist
  MISC_FEATURE (1): Xaa is 4-imidazoacetyl (CA)
  MISC_FEATURE (2): Xaa is 2-aminoisobutyric acid (Aib)
  MISC_FEATURE (16)..(20): amino acids at positions 16 and 20 form a ring
XXQGTFTSDYSICMDEKHQKDFVNWLLNTK

SEQ ID NO: 60 - protein, 30 aa, Artificial Sequence
  Trigonal agonist
  MISC_FEATURE (1): Xaa is 4-imidazoacetyl (CA)
  MISC_FEATURE (2): Xaa is 2-aminoisobutyric acid (Aib)
  MISC_FEATURE (16)..(20): amino acids at positions 16 and 20 form a ring
XXQGTFTSDYSIAMDEKHCKDFVNWLLNTK

SEQ ID NO: 61 - protein, 30 aa, Artificial Sequence
  Trigonal agonist
  MISC_FEATURE (1): Xaa is 4-imidazoacetyl (CA)
  MISC_FEATURE (2): Xaa is 2-aminoisobutyric acid (Aib)
  MISC_FEATURE (16)..(20): amino acids at positions 16 and 20 form a ring
XXQGTFTSDYSIAMDEIACKDFVNWLLNTK

SEQ ID NO: 62 - protein, 39 aa, Artificial Sequence
  Trigonal agonist
  MISC_FEATURE (1): Xaa is 4-imidazoacetyl (CA)
  MISC_FEATURE (2): Xaa is 2-aminoisobutyric acid (Aib)
XXQGTFTSDKSKYLDERAAQDFVQWLLDGGPSSGAPPPS

SEQ ID NO: 63 - protein, 39 aa, Artificial Sequence
  Trigonal agonist
  MISC_FEATURE (1): Xaa is 4-imidazoacetyl (CA)
  MISC_FEATURE (2): Xaa is 2-aminoisobutyric acid (Aib)
XXQGTFTSDCSKYLDERAAQDFVQWLLDGGPSSGAPPPS

SEQ ID NO: 64 - protein, 39 aa, Artificial Sequence
  Trigonal agonist
  MISC_FEATURE (2): Xaa is 2-aminoisobutyric acid (Aib)
  MISC_FEATURE (16)..(20): amino acids at positions 16 and 20 form a ring
YXQGTFTSDYSKYLDECAAKEFVQWLLDHHPSSGQPPPS

SEQ ID NO: 65 - protein, 39 aa, Artificial Sequence
  Trigonal agonist
  MISC_FEATURE (2): Xaa is 2-aminoisobutyric acid (Aib)
  MISC_FEATURE (16)..(20): amino acids at positions 16 and 20 form a ring
HXQGTFTSDYSKCLDEKRAKEFVQWLLDHHPSSGQPPPS

SEQ ID NO: 66 - protein, 39 aa, Artificial Sequence
  Trigonal agonist
  MISC_FEATURE (2): Xaa is 2-aminoisobutyric acid (Aib)
  MISC_FEATURE (16)..(20): amino acids at positions 16 and 20 form a ring
YXQGTFTSDYSKYLDECRAKDFVQWLLDHHPSSGQPPPS

SEQ ID NO: 67 - protein, 39 aa, Artificial Sequence
  Trigonal agonist
  MISC_FEATURE (2): Xaa is 2-aminoisobutyric acid (Aib)
  MISC_FEATURE (16)..(20): amino acids at positions 16 and 20 form a ring
YXQGTFTSDYSKYLDECAAKDFVQWLLDHHPSSGQPPPS

SEQ ID NO: 68 - protein, 39 aa, Artificial Sequence
  Trigonal agonist
  MISC_FEATURE (2): Xaa is 2-aminoisobutyric acid (Aib)
  MISC_FEATURE (16)..(20): amino acids at positions 16 and 20 form a ring
YXQGTFTSDYSKCLDEKAAKEFVQWLLDHHPSSGQPPPS

SEQ ID NO: 69 - protein, 39 aa, Artificial Sequence
  Trigonal agonist
  MISC_FEATURE (2): Xaa is 2-aminoisobutyric acid (Aib)
  MISC_FEATURE (16)..(20): amino acids at positions 16 and 20 form a ring
YXQGTFTSDYSKCLDERAAKEFVQWLLDHHPSSGQPPPS

SEQ ID NO: 70 - protein, 39 aa, Artificial Sequence
  Trigonal agonist
  MISC_FEATURE (2): Xaa is 2-aminoisobutyric acid (Aib)
  MISC_FEATURE (16)..(20): amino acids at positions 16 and 20 form a ring
YXQGTFTSDYSKCLDEKRAKDFVQWLLDHHPSSGQPPPS

SEQ ID NO: 71 - protein, 39 aa, Artificial Sequence
  Trigonal agonist
  MISC_FEATURE (2): Xaa is 2-aminoisobutyric acid (Aib)
  MISC_FEATURE (16)..(20): amino acids at positions 16 and 20 form a ring
YXQGTFTSDYSKYLDERACKDFVQWLLDHHPSSGQPPPS

SEQ ID NO: 72 - protein, 39 aa, Artificial Sequence
  Trigonal agonist
  MISC_FEATURE (2): Xaa is 2-aminoisobutyric acid (Aib)
  MISC_FEATURE (16)..(20): amino acids at positions 16 and 20 form a ring
YXQGTFTSDCSKYLDERAAKDFVQWLLDHHPSSGQPPPS

SEQ ID NO: 73 - protein, 39 aa, Artificial Sequence
  Trigonal agonist
  MISC_FEATURE (1): Xaa is 4-imidazoacetyl (CA)
  MISC_FEATURE (2): Xaa is 2-aminoisobutyric acid (Aib)
  MISC_FEATURE (16)..(20): amino acids at positions 16 and 20 form a ring
XXQGTFTSDYSKYLDECRAKEFVQWLLDHHPSSGQPPPS

SEQ ID NO: 74 - protein, 39 aa, Artificial Sequence
  Trigonal agonist
  MISC_FEATURE (1): Xaa is 4-imidazoacetyl (CA)
  MISC_FEATURE (2): Xaa is 2-aminoisobutyric acid (Aib)
  MISC_FEATURE (16)..(20): amino acids at positions 16 and 20 form a ring
XXQGTFTSDYSKCLDEKRAKEFVQWLLDHHPSSGQPPPS

SEQ ID NO: 75 - protein, 40 aa, Artificial Sequence
  Trigonal agonist
  MISC_FEATURE (2): Xaa is 2-aminoisobutyric acid (Aib)
  MISC_FEATURE (16)..(20): amino acids at positions 16 and 20 form a ring
YXQGTFTSDYSKYLDEKAAKEFVQWLLDHHPSSGQPPPSC

SEQ ID NO: 76 - protein, 40 aa, Artificial Sequence
  Trigonal agonist
  MISC_FEATURE (2): Xaa is 2-aminoisobutyric acid (Aib)
  MISC_FEATURE (16)..(20): amino acids at positions 16 and 20 form a ring
YXQGTFTSDYSKYLDEKRAKDFVQWLLDHHPSSGQPPPSC

SEQ ID NO: 77 - protein, 40 aa, Artificial Sequence
  Trigonal agonist
  MISC_FEATURE (2): Xaa is 2-aminoisobutyric acid (Aib)
  MISC_FEATURE (16)..(20): amino acids at positions 16 and 20 form a ring
YXQGTFTSDYSKYLDEKAAKDFVQWLLDHHPSSGQPPPSC

SEQ ID NO: 78 - protein, 31 aa, Artificial Sequence
  Trigonal agonist
  MISC_FEATURE (2): Xaa is 2-aminoisobutyric acid (Aib)
  MISC_FEATURE (16)..(20): amino acids at positions 16 and 20 form a ring
HXQGTFTSDYSKYLDEKRQKEFVQWLLDTKC

SEQ ID NO: 79 - protein, 31 aa, Artificial Sequence
  Trigonal agonist
  MISC_FEATURE (2): Xaa is 2-aminoisobutyric acid (Aib)
  MISC_FEATURE (16)..(20): amino acids at positions 16 and 20 form a ring
HXEGTFTSDYSIAMDEIHQKDFVNWLLAQKC

SEQ ID NO: 80 - protein, 31 aa, Artificial Sequence
  Trigonal agonist
  MISC_FEATURE (2): Xaa is 2-aminoisobutyric acid (Aib)
  MISC_FEATURE (16)..(20): amino acids at positions 16 and 20 form a ring
HXEGTFTSDYSIAMDEIHQKDFVDWLLAEKC

SEQ ID NO: 81 - protein, 30 aa, Artificial Sequence
  Trigonal agonist
  MISC_FEATURE (1): Xaa is 4-imidazoacetyl (CA)
  MISC_FEATURE (2): Xaa is 2-aminoisobutyric acid (Aib)
  MISC_FEATURE (16)..(20): amino acids at positions 16 and 20 form a ring
XXQGTFTSDYSKYLDEKRQKEFVQWLLNTC

SEQ ID NO: 82 - protein, 30 aa, Artificial Sequence
  Trigonal agonist
  MISC_FEATURE (1): Xaa is 4-imidazoacetyl (CA)
  MISC_FEATURE (2): Xaa is 2-aminoisobutyric acid (Aib)
  MISC_FEATURE (16)..(20): amino acids at positions 16 and 20 form a ring
XXQGTFTSDYSKYLDEKRQKEFVQWLLDTC

SEQ ID NO: 83 - protein, 30 aa, Artificial Sequence
  Trigonal agonist
  MISC_FEATURE (1): Xaa is 4-imidazoacetyl (CA)
  MISC_FEATURE (2): Xaa is 2-aminoisobutyric acid (Aib)
  MISC_FEATURE (16)..(20): amino acids at positions 16 and 20 form a ring
XXEGTFTSDYSIAMDEIHQKDFVNWLLAQC

SEQ ID NO: 84 - protein, 30 aa, Artificial Sequence
  Trigonal agonist
  MISC_FEATURE (1): Xaa is 4-imidazoacetyl (CA)
  MISC_FEATURE (2): Xaa is 2-aminoisobutyric acid (Aib)
  MISC_FEATURE (16)..(20): amino acids at positions 16 and 20 form a ring
XXEGTFTSDYSIAMDEIHQKDFVDWLLAEC

SEQ ID NO: 85 - protein, 30 aa, Artificial Sequence
  Trigonal agonist
  MISC_FEATURE (1): Xaa is 4-imidazoacetyl (CA)
  MISC_FEATURE (2): Xaa is 2-aminoisobutyric acid (Aib)
  MISC_FEATURE (16)..(20): amino acids at positions 16 and 20 form a ring
XXQGTFTSDYSIAMDEIHQKDFVNWLLAQC

SEQ ID NO: 86 - protein, 30 aa, Artificial Sequence
  Trigonal agonist
  MISC_FEATURE (1): Xaa is 4-imidazoacetyl (CA)
  MISC_FEATURE (2): Xaa is 2-aminoisobutyric acid (Aib)
  MISC_FEATURE (16)..(20): amino acids at positions 16 and 20 form a ring
XXQGTFTSDYSKYLDEKRQKEFVNWLLAQC

SEQ ID NO: 87 - protein, 30 aa, Artificial Sequence
  Trigonal agonist
  MISC_FEATURE (1): Xaa is 4-imidazoacetyl (CA)
  MISC_FEATURE (2): Xaa is 2-aminoisobutyric acid (Aib)
  MISC_FEATURE (16)..(20): amino acids at positions 16 and 20 form a ring
XXQGTFTSDYSIAMDEIHQKDFVNWLLNTC

SEQ ID NO: 88 - protein, 31 aa, Artificial Sequence
  Trigonal agonist
  MISC_FEATURE (1): Xaa is 4-imidazoacetyl (CA)
  MISC_FEATURE (2): Xaa is 2-aminoisobutyric acid (Aib)
  MISC_FEATURE (16)..(20): amino acids at positions 16 and 20 form a ring
XXQGTFTSDYSKYLDEKRQKEFVQWLLNTKC

SEQ ID NO: 89 - protein, 31 aa, Artificial Sequence
  Trigonal agonist
  MISC_FEATURE (1): Xaa is 4-imidazoacetyl (CA)
  MISC_FEATURE (2): Xaa is 2-aminoisobutyric acid (Aib)
  MISC_FEATURE (16)..(20): amino acids at positions 16 and 20 form a ring
XXQGTFTSDYSKYLDEKRQKEFVQWLLDTKC

SEQ ID NO: 90 - protein, 31 aa, Artificial Sequence
  Trigonal agonist
  MISC_FEATURE (1): Xaa is 4-imidazoacetyl (CA)
  MISC_FEATURE (2): Xaa is 2-aminoisobutyric acid (Aib)
  MISC_FEATURE (16)..(20): amino acids at positions 16 and 20 form a ring
XXEGTFTSDYSIAMDEIHQKDFVNWLLAQKC

SEQ ID NO: 91 - protein, 31 aa, Artificial Sequence
  Trigonal agonist
  MISC_FEATURE (1): Xaa is 4-imidazoacetyl (CA)
  MISC_FEATURE (2): Xaa is 2-aminoisobutyric acid (Aib)
  MISC_FEATURE (16)..(20): amino acids at positions 16 and 20 form a ring
XXEGTFTSDYSIAMDEIHQKDFVDWLLAEKC

SEQ ID NO: 92 - protein, 31 aa, Artificial Sequence
  Trigonal agonist
  MISC_FEATURE (1): Xaa is 4-imidazoacetyl (CA)
  MISC_FEATURE (2): Xaa is 2-aminoisobutyric acid (Aib)
  MISC_FEATURE (16)..(20): amino acids at positions 16 and 20 form a ring
XXQGTFTSDYSIAMDEIHQKDFVNWLLAQKC

SEQ ID NO: 93 - protein, 31 aa, Artificial Sequence
  Trigonal agonist
  MISC_FEATURE (1): Xaa is 4-imidazoacetyl (CA)
  MISC_FEATURE (2): Xaa is 2-aminoisobutyric acid (Aib)
  MISC_FEATURE (16)..(20): amino acids at positions 16 and 20 form a ring
XXQGTFTSDYSKYLDEKRQKEFVNWLLAQKC

SEQ ID NO: 94 - protein, 31 aa, Artificial Sequence
  Trigonal agonist
  MISC_FEATURE (1): Xaa is 4-imidazoacetyl (CA)
  MISC_FEATURE (2): Xaa is 2-aminoisobutyric acid (Aib)
  MISC_FEATURE (16)..(20): amino acids at positions 16 and 20 form a ring
XXQGTFTSDYSIAMDEIHQKDFVNWLLNTKC

SEQ ID NO: 95 - protein, 39 aa, Artificial Sequence
  Trigonal agonist
  MISC_FEATURE (2): Xaa is 2-aminoisobutyric acid (Aib)
  MISC_FEATURE (16)..(20): amino acids at positions 16 and 20 form a ring
YXQGTFTSDYSKYLDEKRAKEFVQWLLCHHPSSGQPPPS

SEQ ID NO: 96 - protein, 39 aa, Artificial Sequence
  Trigonal agonist
  MISC_FEATURE (2): Xaa is 2-aminoisobutyric acid (Aib)
  MISC_FEATURE (16)..(20): amino acids at positions 16 and 20 form a ring
YXQGTFTSDYSKYLDEKRAKEFVQWLLDHCPSSGQPPPS

SEQ ID NO: 97 - protein, 39 aa, Artificial Sequence
  Trigonal agonist
  MISC_FEATURE (2): Xaa is 2-aminoisobutyric acid (Aib)
  MISC_FEATURE (16)..(20): amino acids at positions 16 and 20 form a ring
YXQGTFTSDYSKYLDEKRAKEFVQWLLDCHPSSGQPPPS

SEQ ID NO: 98 - protein, 40 aa, Artificial Sequence
  Trigonal agonist
  MISC_FEATURE (2): Xaa is 2-aminoisobutyric acid (Aib)
  MISC_FEATURE (16)..(20): amino acids at positions 16 and 20 form a ring
YXQGTFTSDYSKALDEKAAKEFVNWLLDHHPSSGQPPPSC

SEQ ID NO: 99 - protein, 40 aa, Artificial Sequence
  Trigonal agonist
  MISC_FEATURE (2): Xaa is 2-aminoisobutyric acid (Aib)
  MISC_FEATURE (16)..(20): amino acids at positions 16 and 20 form a ring
YXQGTFTSDYSKALDEKAAKDFVNWLLDHHPSSGQPPPSC

SEQ ID NO: 100 - protein, 40 aa, Artificial Sequence
  Trigonal agonist
  MISC_FEATURE (2): Xaa is 2-aminoisobutyric acid (Aib)
  MISC_FEATURE (16)..(20): amino acids at positions 16 and 20 form a ring
YXQGTFTSDYSKALDEKAAKEFVQWLLDQHPSSGQPPPSC

SEQ ID NO: 101 - protein, 40 aa, Artificial Sequence
  Trigonal agonist
  MISC_FEATURE (2): Xaa is 2-aminoisobutyric acid (Aib)
  MISC_FEATURE (16)..(20): amino acids at positions 16 and 20 form a ring
YXQGTFTSDYSKALDEKAAKEFVNWLLDQHPSSGQPPPSC

SEQ ID NO: 102 - protein, 40 aa, Artificial Sequence
  Trigonal agonist
  MISC_FEATURE (2): Xaa is 2-aminoisobutyric acid (Aib)
  MISC_FEATURE (16)..(20): amino acids at positions 16 and 20 form a ring
YXQGTFTSDYSKALDEKAAKDFVNWLLDQHPSSGQPPPSC

SEQ ID NO: 103 - protein, 30 aa, Artificial Sequence
  General Formula 1
  MISC_FEATURE (1): Xaa is His (H), 4-imidazoacetyl (CA), or Tyr (Y)
  MISC_FEATURE (2): Xaa is Gly (G), alpha-methyl-glutamic acid, or Aib (2-aminoisobutyric acid)
  MISC_FEATURE (3): Xaa is Glu (E) or Gln (Q)
  MISC_FEATURE (7): Xaa is Thr (T) or Ile (I)
  MISC_FEATURE (10): Xaa is Leu (L), Tyr (Y), Lys (K), Cys (C), or Val (V)
  MISC_FEATURE (12): Xaa is Lys (K), Ser (S), or Ile (I)
  MISC_FEATURE (13): Xaa is Gln (Q), Tyr (Y), Ala (A), or Cys (C)
  MISC_FEATURE (14): Xaa is Leu (L), Met (M), or Tyr (Y)
  MISC_FEATURE (15): Xaa is Cys (C), Asp (D), Glu (E), or Leu (L)
  MISC_FEATURE (16): Xaa is Gly (G), Glu (E), or Ser (S)
  MISC_FEATURE (17): Xaa is Gln (Q), Arg (R), Ile (I), Glu (E), Cys (C), or Lys (K)
  MISC_FEATURE (18): Xaa is Ala (A), Gln (Q), Arg (R), or His (H)
  MISC_FEATURE (19): Xaa is Ala (A), Gln (Q), Cys (C), or Val (V)
  MISC_FEATURE (20): Xaa is Lys (K), Gln (Q), or Arg (R)
  MISC_FEATURE (21): Xaa is Glu (E), Gln (Q), Leu (L), Cys (C), or Asp (D)
  MISC_FEATURE (23): Xaa is Ile (I) or Val (V)
  MISC_FEATURE (24): Xaa is Ala (A), Gln (Q), Cys (C), Asn (N), Asp (D), or Glu (E)
  MISC_FEATURE (27): Xaa is Val (V), Leu (L), Lys (K), or Met (M)
  MISC_FEATURE (28): Xaa is Cys (C), Lys (K), Ala (A), Asn (N), or Asp (D)
  MISC_FEATURE (29): Xaa is Cys (C), Gly (G), Gln (Q), Thr (T), Glu (E), or His (H)
  MISC_FEATURE (30): Xaa is Cys (C), Gly (G), Lys (K), or His (H), or is absent; and Xaa can be further linked to R1, wherein R1 is Cys (C), GKKNDWKHNIT, m-SSGAPPPS-n, or m-SSGQPPPS-n, or is absent, and wherein m is -Cys-, -Pro-, or -Gly-Pro-, and n is -Cys-, -Gly-, -Ser-, -His-Gl
XXXGTFXSDXSXXXXXXXXXXFXXWLXXXX

SEQ ID NO: 104 - protein, 40 aa, Artificial Sequence
  General Formula 2
  MISC_FEATURE (1): Xaa is His (H), 4-imidazoacetyl (CA), or Tyr (Y)
  MISC_FEATURE (2): Xaa is Gly (G), alpha-methyl-glutamic acid, or Aib (2-aminoisobutyric acid)
  MISC_FEATURE (10): Xaa is Tyr (Y) or Cys (C)
  MISC_FEATURE (13): Xaa is Gln (Q), Tyr (Y), Ala (A), or Cys (C)
  MISC_FEATURE (14): Xaa is Leu (L), Met (M), or Tyr (Y)
  MISC_FEATURE (15): Xaa is Asp (D), Glu (E), or Leu (L)
  MISC_FEATURE (16): Xaa is Gly (G), Glu (E), or Ser (S)
  MISC_FEATURE (17): Xaa is Gln (Q), Arg (R), Ile (I), Glu (E), Cys (C), or Lys (K)
  MISC_FEATURE (18): Xaa is Ala (A), Gln (Q), Arg (R), or His (H)
  MISC_FEATURE (19): Xaa is Ala (A), Gln (Q), Cys (C), or Val (V)
  MISC_FEATURE (20): Xaa is Lys (K), Gln (Q), or Arg (R)
  MISC_FEATURE (21): Xaa is Glu (E), Gln (Q), Leu (L), Cys (C), or Asp (D)
  MISC_FEATURE (23): Xaa is Ile (I) or Val (V)
  MISC_FEATURE (24): Xaa is Ala (A), Gln (Q), Cys (C), Asn (N), or Glu (E)
  MISC_FEATURE (28): Xaa is Cys (C), Lys (K), Asn (N), or Asp (D)
  MISC_FEATURE (29): Xaa is Cys (C), Gly (G), Gln (Q), or His (H)
  MISC_FEATURE (30): Xaa is Cys (C), Gly (G), Lys (K), or His (H)
  MISC_FEATURE (31): Xaa is Pro (P) or Cys (C)
  MISC_FEATURE (40): Xaa is Cys (C), or is absent
XXQGTFTSDXSKXXXXXXXXXFXXWLLXXXXSSGQPPPSX

SEQ ID NO: 105 - protein, 40 aa, Artificial Sequence
  General Formula 3
  MISC_FEATURE (1): Xaa is His (H) or Tyr (Y)
  MISC_FEATURE (2): Xaa is alpha-methyl-glutamic acid, or Aib (2-aminoisobutyric acid)
  MISC_FEATURE (13): Xaa is Tyr (Y), Ala (A), or Cys (C)
  MISC_FEATURE (17): Xaa is Arg (R), Cys (C), or Lys (K)
  MISC_FEATURE (18): Xaa is Ala (A) or Arg (R)
  MISC_FEATURE (19): Xaa is Ala (A) or Cys (C)
  MISC_FEATURE (21): Xaa is Glu (E) or Asp (D)
  MISC_FEATURE (24): Xaa is Gln (Q) or Asn (N)
  MISC_FEATURE (28): Xaa is Cys (C) or Asp (D)
  MISC_FEATURE (29): Xaa is Cys (C), Gln (Q), or His (H)
  MISC_FEATURE (30): Xaa is Cys (C) or His (H)
  MISC_FEATURE (31): Xaa is Pro (P) or Cys (C)
  MISC_FEATURE (40): Xaa is Cys (C), or is absent
XXQGTFTSDYSKXLDEXXXKXFVXWLLXXXXSSGQPPPSX

SEQ ID NO: 106 - protein, 11 aa, Artificial Sequence
  R1
GKKNDWKHNIT

SEQ ID NO: 107 - protein, 8 aa, Artificial Sequence
  R1
SSGAPPPS

SEQ ID NO: 108 - protein, 8 aa, Artificial Sequence
  R1
SSGQPPPS

SEQ ID NO: 109 - protein, 9 aa, Artificial Sequence
  R1
CSSGQPPPS

SEQ ID NO: 110 - protein, 11 aa, Artificial Sequence
  R1
PSSGAPPPSHG

SEQ ID NO: 111 - protein, 11 aa, Artificial Sequence
  R1
GPSSGAPPPSC

SEQ ID NO: 112 - protein, 9 aa, Artificial Sequence
  R1
PSSGAPPPS

SEQ ID NO: 113 - protein, 10 aa, Artificial Sequence
  R1
PSSGAPPPSG

SEQ ID NO: 114 - protein, 11 aa, Artificial Sequence
  R1
PSSGAPPPSHG

SEQ ID NO: 115 - protein, 10 aa, Artificial Sequence
  R1
PSSGAPPPSS

SEQ ID NO: 116 - protein, 9 aa, Artificial Sequence
  R1
PSSGQPPPS

SEQ ID NO: 117 - protein, 10 aa, Artificial Sequence
  R1
PSSGQPPPSC

SEQ ID NO: 118 - protein, 12 aa, HOMO SAPIENS
ESKYGPPCPSCP

SEQ ID NO: 119 - protein, 11 aa, Artificial Sequence
  Variant of hinge region
ESKYGPPPSCP

SEQ ID NO: 120 - protein, 11 aa, Artificial Sequence
  Variant of hinge region
ESKYGPPCPSP

SEQ ID NO: 121 - protein, 10 aa, Artificial Sequence
  Variant of hinge region
ESKYGPPCPS

SEQ ID NO: 122 - protein, 10 aa, Artificial Sequence
  Variant of hinge region
ESKYGPPCPP

SEQ ID NO: 123 - protein, 8 aa, Artificial Sequence
  Variant of hinge region
KYGPPCPS

SEQ ID NO: 124 - protein, 8 aa, Artificial Sequence
  Variant of hinge region
ESKYGPPC

SEQ ID NO: 125 - protein, 7 aa, Artificial Sequence
  Variant of hinge region
EKYGPPC

SEQ ID NO: 126 - protein, 6 aa, Artificial Sequence
  Variant of hinge region
ESPSCP

SEQ ID NO: 127 - protein, 5 aa, Artificial Sequence
  Variant of hinge region
EPSCP

SEQ ID NO: 128 - protein, 4 aa, Artificial Sequence
  Variant of hinge region
PSCP

SEQ ID NO: 129 - protein, 10 aa, Artificial Sequence
  Variant of hinge region
ESKYGPPSCP

SEQ ID NO: 130 - protein, 9 aa, Artificial Sequence
  Variant of hinge region
KYGPPPSCP

SEQ ID NO: 131 - protein, 9 aa, Artificial Sequence
  Variant of hinge region
ESKYGPSCP

SEQ ID NO: 132 - protein, 8 aa, Artificial Sequence
  Variant of hinge region
ESKYGPPC

SEQ ID NO: 133 - protein, 7 aa, Artificial Sequence
  Variant of hinge region
KYGPPCP

SEQ ID NO: 134 - protein, 7 aa, Artificial Sequence
  Variant of hinge region
ESKPSCP

SEQ ID NO: 135 - protein, 6 aa, Artificial Sequence
  Variant of hinge region
ESPSCP

SEQ ID NO: 136 - protein, 4 aa, Artificial Sequence
  Variant of hinge region
EPSC

SEQ ID NO: 137 - protein, 3 aa, Artificial Sequence
  Variant of hinge region
SCP

SEQ ID NO: 138 - protein, 221 aa, homo sapiens
PSCPAPEFLGGPSVFLFPPKPKDTLMISRTPEVTCVVVDVSQEDPEVQFNWYVDGVEVHNAKTKPREEQFNSTYRVVSVLTVLHQDWLNGKEYKCKVSNKGLPSSIEKTISKAKGQPREPQVYTLPPSQEEMTKNQVSLTCLVKGFYPSDIAVEWESNGQPENNYKTTPPVLDSDGSFFLYSRLTVDKSRWQEGNVFSCSVMHEALHNHYTQKSLSLSLGK

SEQ ID NO: 139 - protein, 442 aa, Homo sapiens
  MISC_FEATURE (1)..(442): Amino acids at position 1 to 442 form Human Immunoglobulin G4 Fc Fragment (homodimer)
  MISC_FEATURE (1)..(221): Amino acids at position 1 to 221 form one monomer
  MISC_FEATURE (222)..(442): Amino acids at position 222 to 442 form one monomer
  DISULFID (3)..(224): Amino acids at position 3 and position 224 form an inter-disulfide bond
  DISULFID (35)..(95): Amino acids at position 35 and position 95 form an intra-chain disulfide bond
  DISULFID (141)..(199): Amino acids at position 141 and position 199 form an intra-chain disulfide bond
  DISULFID (256)..(316): Amino acids at position 256 and position 316 form an intra-chain disulfide bond
  DISULFID (362)..(420): Amino acids at position 362 and position 420 form an intra-chain disulfide bond
PSCPAPEFLGGPSVFLFPPKPKDTLMISRTPEVTCVVVDVSQEDPEVQFNWYVDGVEVHNAKTKPREEQFNSTYRVVSVLTVLHQDWLNGKEYKCKVSNKGLPSSIEKTISKAKGQPREPQVYTLPPSQEEMTKNQVSLTCLVKGFYPSDIAVEWESNGQPENNYKTTPPVLDSDGSFFLYSRLTVDKSRWQEGNVFSCSVMHEALHNHYTQKSLSLSLGKPSCPAPEFLGGPSVFLFPPKPKDTLMISRTPEVTCVVVDVSQEDPEVQFNWYVDGVEVHNAKTKPREEQFNSTYRVVSVLTVLHQDWLNGKEYKCKVSNKGLPSSIEKTISKAKGQPREPQVYTLPPSQEEMTKNQVSLTCLVKGFYPSDIAVEWESNGQPENNYKTTPPVLDSDGSFFLYSRLTVDKSRWQEGNVFSCSVMHEALHNHYTQKSLSLSLGK